European Patent Specification EP 3 884 041 B1, published September 2, 2026. Title: METHODS FOR EXPANSION OF NATURAL KILLER (NK) CELL SUBSET AND RELATED COMPOSITIONS AND METHODS. Applicant: Indapta Therapeutics, Inc Bigley, Austin. Application Not yet assigned. The sequence listing filed with the application follows.

SEQUENCE LISTING (18 sequences)

SEQ ID NO: 1 - protein, 86 aa, Homo sapiens
  High affinity immunoglobulin gamma Fc receptor I
MIPAVVLLLLLLVEQAAALGEPQLCYILDAILFLYGIVLTLLYCRLKIQVRKAAITSYEKSDGVYTGLSTRNQETYETLKHEKPPQ

SEQ ID NO: 2 - DNA, 21 bp, Artificial Sequence
  PCR primer
atatttacagaatggcacagg

SEQ ID NO: 3 - DNA, 20 bp, Artificial Sequence
  PCR primer
gacttggtacccaggttgaa

SEQ ID NO: 4 - DNA, 32 bp, Artificial Sequence
  PCR primer
atcagattcgatcctacttctgcagggggcat

SEQ ID NO: 5 - DNA, 32 bp, Artificial Sequence
  PCR primer
acgtgctgagcttgagtgatggtgatgttcac

SEQ ID NO: 6 - DNA, 24 bp, Artificial Sequence
  PCR primer
cccaactcaacttcccagtgtgat

SEQ ID NO: 7 - DNA, 30 bp, Artificial Sequence
  PCR primer
gaaatctaccttttcctctaatagggcaat

SEQ ID NO: 8 - DNA, 29 bp, Artificial Sequence
  PCR primer
gaaatctaccttttcctctaatagggcaa

SEQ ID NO: 9 - DNA, 28 bp, Artificial Sequence
  PCR primer
gaaatctaccttttcctctaatagggca

SEQ ID NO: 10 - DNA, 21 bp, Artificial Sequence
  CD16 sense primer
ccaaaagccacactcaaagac

SEQ ID NO: 11 - DNA, 21 bp, Artificial Sequence
  CD16 antisense primer
acccaggtggaaagaatgatg

SEQ ID NO: 12 - DNA, 25 bp, Artificial Sequence
  TaqMan probe
aacatcaccatcactcaaggtttgg

SEQ ID NO: 13 - DNA, 25 bp, Artificial Sequence
  V allele forward primer
ctgaagacacatttttactcccaaa

SEQ ID NO: 14 - DNA, 22 bp, Artificial Sequence
  V allele reverse primer
tccaaaagccacactcaaagac

SEQ ID NO: 15 - DNA, 25 bp, Artificial Sequence
  F allele forward primer
ctgaagacacatttttactcccaac

SEQ ID NO: 16 - protein, 238 aa, Homo sapiens
  CD16 (F158)
GMRTEDLPKAVVFLEPQWYRVLEKDSVTLKCQGAYSPEDNSTQWFHNESLISSQASSYFIDAATVDDSGEYRCQTNLSTLSDPVQLEVHIGWLLLQAPRWVFKEEDPIHLRCHSWKNTALHKVTYLQNGKGRKYFHHNSDFYIPKATLKDSGSYFCRGLFGSKNVSSETVNITITQGLAVSTISSFFPPGYQVSFCLVMVLLFAVDTGLYFSVKTNIRSSTRDWKDHKFKWRKDPQDK

SEQ ID NO: 17 - protein, 16 aa, Artificial Sequence
  Signal peptide
MWQLLLPTALLLLVSA

SEQ ID NO: 18 - protein, 238 aa, Homo sapiens
  CD16 VAR_003960
GMRTEDLPKAVVFLEPQWYRVLEKDSVTLKCQGAYSPEDNSTQWFHNESLISSQASSYFIDAATVDDSGEYRCQTNLSTLSDPVQLEVHIGWLLLQAPRWVFKEEDPIHLRCHSWKNTALHKVTYLQNGKGRKYFHHNSDFYIPKATLKDSGSYFCRGLVGSKNVSSETVNITITQGLAVSTISSFFPPGYQVSFCLVMVLLFAVDTGLYFSVKTNIRSSTRDWKDHKFKWRKDPQDK